European Patent Specification EP 3 331 563 B1, published April 19, 2023. Title: Anti-CD154 antibodies and methods of using them. Applicant: Janssen Biotech, Inc. Fransson, Johan Leu, Jocelyn Obmolova, Galina Suri, Anish Teng, Fang Teplyakov, Alexey Zhou, Hong. Application To Be Assigned. The sequence listing filed with the application follows.

SEQUENCE LISTING (87 sequences)

SEQ ID NO: 1 - protein, 261 aa, Homo sapiens
MIETYNQTSPRSAATGLPISMKIFMYLLTVFLITQMIGSALFAVYLHRRLDKIEDERNLHEDFVFMKTIQRCNTGERSLSLLNCEEIKSQFEGFVKDIMLNKEETKKENSFEMQKGDQNPQIAAHVISEASSKTTSVLQWAEKGYYTMSNNLVTLENGKQLTVKRQGLYYIYAQVTFCSNREASSQAPFIASLCLKSPGRFERILLRAANTHSSAKPCGQQSIHLGGVFELQPGASVFVNVTDPSQVSHGTGFTSFGLLKL

SEQ ID NO: 2 - protein, 261 aa, Callithrix jacchus
MIETYNQPVPRSAATGPPVSMKIFMYLLTVFLITQMIGSALFAVYLHRRLDKIEDERNLHEDFVFMKTIQRCNTGERSLSLLNCEEIKSQFEGFVKDIMLNKEEKKKENSFEMQKGDQNPQIAAHVISEASSKTTSVLQWAEKGYYTMSNNLVTLENGKQLTVKRQGLYYIYAQVTFCSNREASSQAPFIASLCLKPPNRFERILLRAANTHSSAKPCGQQSIHLGGIFELQPGASVFVNVTDPSQVSHGTGFTSFGLLKL

SEQ ID NO: 3 - protein, 261 aa, Macaca fascicularis
MIETYNQPSPRSAATGLPVRMKIFMYLLTIFLITQMIGSALFAVYLHRRLDKIEDERNLHEDFVFMKTIQRCNTGERSLSLLNCEEIKSQFEGFVKDIMLNKEEKKKENSFEMQKGDQNPQIAAHVISEASSKTTSVLQWAEKGYYTMSNNLVTLENGKQLTVKRQGLYYIYAQVTFCSNREASSQAPFIASLCLKSPGRFERILLRAANTHSSAKPCGQQSIHLGGVFELQPGASVFVNVTDPSQVSHGTGFTSFGLLKL

SEQ ID NO: 4 - protein, 149 aa, Homo sapiens
MQKGDQNPQIAAHVISEASSKTTSVLQWAEKGYYTMSNNLVTLENGKQLTVKRQGLYYIYAQVTFCSNREASSQAPFIASLCLKSPGRFERILLRAANTHSSAKPCGQQSIHLGGVFELQPGASVFVNVTDPSQVSHGTGFTSFGLLKL

SEQ ID NO: 5 - protein, 149 aa, Callithrix jacchus
MQKGDQNPQIAAHVISEASSKTTSVLQWAEKGYYTMSNNLVTLENGKQLTVKRQGLYYIYAQVTFCSNREASSQAPFIASLCLKPPNRFERILLRAANTHSSAKPCGQQSIHLGGIFELQPGASVFVNVTDPSQVSHGTGFTSFGLLKL

SEQ ID NO: 6 - protein, 149 aa, Macaca fascicularis; identical to SEQ ID NO: 4

SEQ ID NO: 7 - protein, 161 aa, Artificial Sequence
  Fusion protein shCD154-Histag
GSHHHHHHGGGSMQKGDQNPQIAAHVISEASSKTTSVLQWAEKGYYTMSNNLVTLENGKQLTVKRQGLYYIYAQVTFCSNREASSQAPFIASLCLKSPGRFERILLRAANTHSSAKPCGQQSIHLGGVFELQPGASVFVNVTDPSQVSHGTGFTSFGLLKL

SEQ ID NO: 8 - protein, 161 aa, Artificial Sequence
  Fusion protein smCD154-histag
GSHHHHHHGGGSMQKGDQNPQIAAHVISEASSKTTSVLQWAEKGYYTMSNNLVTLENGKQLTVKRQGLYYIYAQVTFCSNREASSQAPFIASLCLKPPNRFERILLRAANTHSSAKPCGQQSIHLGGIFELQPGASVFVNVTDPSQVSHGTGFTSFGLLKL

SEQ ID NO: 9 - protein, 161 aa, Artificial Sequence; identical to SEQ ID NO: 7
  Fusion protein scCD154-histag

SEQ ID NO: 10 - protein, 6 aa, Artificial Sequence
  His6 tag
HHHHHH

SEQ ID NO: 11 - protein, 33 aa, Artificial Sequence
  ILZ tag
RMKQIEDKIEEILSKIYHIENEIARIKKLIGER

SEQ ID NO: 12 - protein, 198 aa, Artificial Sequence
  Fusion protein shCD154-ILZ
GSHHHHHHGGGSRMKQIEDKIEEILSKIYHIENEIARIKKLIGERGGGSMQKGDQNPQIAAHVISEASSKTTSVLQWAEKGYYTMSNNLVTLENGKQLTVKRQGLYYIYAQVTFCSNREASSQAPFIASLCLKSPGRFERILLRAANTHSSAKPCGQQSIHLGGVFELQPGASVFVNVTDPSQVSHGTGFTSFGLLKL

SEQ ID NO: 13 - protein, 198 aa, Artificial Sequence
  Fusion protein smCD154-ILZ
GSHHHHHHGGGSRMKQIEDKIEEILSKIYHIENEIARIKKLIGERGGGSMQKGDQNPQIAAHVISEASSKTTSVLQWAEKGYYTMSNNLVTLENGKQLTVKRQGLYYIYAQVTFCSNREASSQAPFIASLCLKPPNRFERILLRAANTHSSAKPCGQQSIHLGGIFELQPGASVFVNVTDPSQVSHGTGFTSFGLLKL

SEQ ID NO: 14 - protein, 198 aa, Artificial Sequence; identical to SEQ ID NO: 12
  Fusion protein scCD154-ILZ

SEQ ID NO: 15 - protein, 277 aa, Homo sapiens
MVRLPLQCVLWGCLLTAVHPEPPTACREKQYLINSQCCSLCQPGQKLVSDCTEFTETECLPCGESEFLDTWNRETHCHQHKYCDPNLGLRVQQKGTSETDTICTCEEGWHCTSEACESCVLHRSCSPGFGVKQIATGVSDTICEPCPVGFFSNVSSAFEKCHPWTSCETKDLVVQQAGTNKTDVVCGPQDRLRALVVIPIIFGILFAILLVLVFIKKVAKKPTNKAPHPKQEPQEINFPDDLPGSNTAAPVQETLHGCQPVTQEDGKESRISVQERQ

SEQ ID NO: 16 - protein, 5 aa, Artificial Sequence
  HCDR1
SYAIS

SEQ ID NO: 17 - protein, 5 aa, Artificial Sequence
  HCDR1
SYGIS

SEQ ID NO: 18 - protein, 7 aa, Artificial Sequence
  HCDR1
SYSFYWG

SEQ ID NO: 19 - protein, 5 aa, Artificial Sequence
  HCDR1
AYYIH

SEQ ID NO: 20 - protein, 5 aa, Artificial Sequence
  HCDR1
DYYIH

SEQ ID NO: 21 - protein, 7 aa, Artificial Sequence
  HCDR1
SFIYYWG

SEQ ID NO: 22 - protein, 17 aa, Artificial Sequence
  HCDR2
GIIPIFGTANYAQKFQG

SEQ ID NO: 23 - protein, 17 aa, Artificial Sequence
  HCDR2
WISPIFGNTNYAQKFQG

SEQ ID NO: 24 - protein, 17 aa, Artificial Sequence
  HCDR2
GISPYFGNTNYAQKFQG

SEQ ID NO: 25 - protein, 16 aa, Artificial Sequence
  HCDR2
SLYYSGSTYYNPSLKS

SEQ ID NO: 26 - protein, 17 aa, Artificial Sequence
  HCDR2
RINPDSGGTDYAQRFQG

SEQ ID NO: 27 - protein, 17 aa, Artificial Sequence
  HCDR2
RFNPNSGDTNGAQKFQG

SEQ ID NO: 28 - protein, 16 aa, Artificial Sequence
  HCDR2
CIYSSGGTYYNPSLKS

SEQ ID NO: 29 - protein, 14 aa, Artificial Sequence
  HCDR3
GASVWDGPAEVFDY

SEQ ID NO: 30 - protein, 9 aa, Artificial Sequence
  HCDR3
SRYYGDLDY

SEQ ID NO: 31 - protein, 12 aa, Artificial Sequence
  HCDR3
DTGWVGAFYLDY

SEQ ID NO: 32 - protein, 12 aa, Artificial Sequence
  HCDR3
LQLGTTTDYFDH

SEQ ID NO: 33 - protein, 20 aa, Artificial Sequence
  HCDR3
DWNYYDGSGYFGPGYYGLDV

SEQ ID NO: 34 - protein, 11 aa, Artificial Sequence
  HCDR3
EGELAGIFFDY

SEQ ID NO: 35 - protein, 12 aa, Artificial Sequence
  HCDR3
LWLGTTTDYFDY

SEQ ID NO: 36 - protein, 17 aa, Artificial Sequence
  LCDR1
KSSQSVLASSNNENFLA

SEQ ID NO: 37 - protein, 11 aa, Artificial Sequence
  LCDR1
RASQSISSYLN

SEQ ID NO: 38 - protein, 17 aa, Artificial Sequence
  LCDR1
KSSQSVLYSSNNKNYLA

SEQ ID NO: 39 - protein, 11 aa, Artificial Sequence
  LCDR1
SGDELGDKFAC

SEQ ID NO: 40 - protein, 11 aa, Artificial Sequence
  LCDR1
SGDKLGDKYVC

SEQ ID NO: 41 - protein, 11 aa, Artificial Sequence
  LCDR1
SGDKLGDKYVS

SEQ ID NO: 42 - protein, 11 aa, Artificial Sequence
  LCDR1
SGDKLGDKFAC

SEQ ID NO: 43 - protein, 7 aa, Artificial Sequence
  LCDR2
SASTRES

SEQ ID NO: 44 - protein, 7 aa, Artificial Sequence
  LCDR2
YANSLQS

SEQ ID NO: 45 - protein, 7 aa, Artificial Sequence
  LCDR2
WASTRES

SEQ ID NO: 46 - protein, 7 aa, Artificial Sequence
  LCDR2
QENKRPS

SEQ ID NO: 47 - protein, 7 aa, Artificial Sequence
  LCDR2
QDRKRPS

SEQ ID NO: 48 - protein, 7 aa, Artificial Sequence
  LCDR2
QDDKRPS

SEQ ID NO: 49 - protein, 7 aa, Artificial Sequence
  LCDR2
YASSLQS

SEQ ID NO: 50 - protein, 7 aa, Artificial Sequence
  LCDR2
YANTLQS

SEQ ID NO: 51 - protein, 9 aa, Artificial Sequence
  LCDR3
QQAYTTPFT

SEQ ID NO: 52 - protein, 9 aa, Artificial Sequence
  LCDR3
QQSDSIPWT

SEQ ID NO: 53 - protein, 9 aa, Artificial Sequence
  LCDR3
QQYYSTPLT

SEQ ID NO: 54 - protein, 9 aa, Artificial Sequence
  LCDR3
QAWDSDTAV

SEQ ID NO: 55 - protein, 9 aa, Artificial Sequence
  LCDR3
QAWDSGTVV

SEQ ID NO: 56 - protein, 9 aa, Artificial Sequence
  LCDR3
QAWDSSTVV

SEQ ID NO: 57 - protein, 9 aa, Artificial Sequence
  LCDR3
QAWDSNTVV

SEQ ID NO: 58 - protein, 123 aa, Artificial Sequence
  VH of C4LB5
QVQLVQSGAEVKKPGSSVKVSCKASGGTFSSYAISWVRQAPGQGLEWMGGIIPIFGTANYAQKFQGRVTITADESTSTAYMELSSLRSEDTAVYYCARGASVWDGPAEVFDYWGQGTLVTVSS

SEQ ID NO: 59 - protein, 118 aa, Artificial Sequence
  VH of C4LB89
QVQLVQSGAEVKKPGSSVKVSCKASGGTFSSYGISWVRQAPGQGLEWMGWISPIFGNTNYAQKFQGRVTITADESTSTAYMELSSLRSEDTAVYYCARSRYYGDLDYWGQGTLVTVSS

SEQ ID NO: 60 - protein, 121 aa, Artificial Sequence
  VH of C4LB94
QVQLVQSGAEVKKPGSSVKVSCKASGGTFSSYAISWVRQAPGQGLEWMGGISPYFGNTNYAQKFQGRVTITADESTSTAYMELSSLRSEDTAVYYCARDTGWVGAFYLDYWGQGTLVTVSS

SEQ ID NO: 61 - protein, 122 aa, Artificial Sequence
  VH of C4LB150
QLQLQESGPGLVKPSETLSLTCTVSGGSISSYSFYWGWIRQPPGQGLEWIGSLYYSGSTYYNPSLKSRATMSVVTSKTQFSLNLNSVTAADTAVYYCARLQLGTTTDYFDHWGQGTLVTVSS

SEQ ID NO: 62 - protein, 129 aa, Artificial Sequence
  VH of C4LB189
QVQLVQSGAEVKKPGASVKVSCKASGYTFAAYYIHWVRQAPGQGLEWMGRINPDSGGTDYAQRFQGRVTMTRDTSISTAYMELSRLRSDDTAVFYCARDWNYYDGSGYFGPGYYGLDVWGQGTTVTVSS

SEQ ID NO: 63 - protein, 120 aa, Artificial Sequence
  VH of C4LB191
QVQLVQSGAEVKKPGASMKVSCKASGYTFTDYYIHWVRQAPGQGLEWVGRFNPNSGDTNGAQKFQGRVTMTRDTSISTAYMELTRLRSDDTAVYHCAREGELAGIFFDYWGQGTLVTVSS

SEQ ID NO: 64 - protein, 122 aa, Artificial Sequence
  VH of C4LB199
QVQLQESGPGLVKPSETLSLTCTVSGDSISSFIYYWGWIRQPPGKGLDWVGCIYSSGGTYYNPSLKSRVTISVDTSKNQFSLKLPSVTAADTAVYYCARLWLGTTTDYFDYWGQGTLVTVSS

SEQ ID NO: 65 - protein, 113 aa, Artificial Sequence
  VL of C4LB5
DIVMTQSPDSLAVSLGERATINCKSSQSVLASSNNENFLAWYQQKPGQPPKLLIYSASTRESGVPDRFSGSGSGTDFTLTISSLQAEDVAVYYCQQAYTTPFTFGQGTKVEIK

SEQ ID NO: 66 - protein, 107 aa, Artificial Sequence
  VL of C4LB89
DIQMTQSPSSLSASVGDRVTITCRASQSISSYLNWYQQKPGKAPKLLIYYANSLQSGVPSRFSGSGSGTDFTLTISSLQPEDFATYYCQQSDSIPWTFGQGTKVEIK

SEQ ID NO: 67 - protein, 113 aa, Artificial Sequence
  VL of C4LB94
DIVMTQSPDSLAVSLGERATINCKSSQSVLYSSNNKNYLAWYQQKPGQPPKLLIYWASTRESGVPDRFSGSGSGTDFTLTISSLQAEDVAVYYCQQYYSTPLTFGQGTKVEIK

SEQ ID NO: 68 - protein, 106 aa, Artificial Sequence
  VL of C4LB150
SYELTQPPSVSVSPGQTASITCSGDELGDKFACWYQQKPGQSPVLVIWQENKRPSGIPERFSGSNSGNTATLTISGTQAMDEADYYCQAWDSDTAVFGGGTKLTVL

SEQ ID NO: 69 - protein, 106 aa, Artificial Sequence
  VL of C4LB189
SYELTQPPSVSVSPGQTASVTCSGDKLGDKYVCWYQRKPGQSPVLVIYQDRKRPSGIPERFSGSNSGNTATLTISGTQAIDEADYYCQAWDSGTVVFGRGTKLTVL

SEQ ID NO: 70 - protein, 106 aa, Artificial Sequence
  VL of C4LB191
SYELTQPPSVSVSPGQTASITCSGDKLGDKYVSWNHQKPGQSPVLVIYQDRKRPSGIPERFSGSNSGNTATLTISGTQAMDEADYYCQAWDSSTVVFGGGTKLTVL

SEQ ID NO: 71 - protein, 106 aa, Artificial Sequence
  VL of C4LB199
SYELTQPPSVSVSPGQTVSITCSGDKLGDKFACWYQQKPGQSPVVVIYQDDKRPSGIPERFSGSTSGNTATLTISGTQAMDEADYYCQAWDSNTVVFGGGTKLTVL

SEQ ID NO: 72 - protein, 107 aa, Artificial Sequence
  VL or C4LB235
DIQMTQSPSSLSASVGDRVTITCRASQSISSYLNWYQQKPGKAPKLLIYYASSLQSGVPSRFSGSGSGTDFTLTISSLQPEDFATYYCQQSDSIPWTFGQGTKVEIK

SEQ ID NO: 73 - protein, 107 aa, Artificial Sequence
  VL of C4LB236
DIQMTQSPSSLSASVGDRVTITCRASQSISSYLNWYQQKPGKAPKLLIYYANTLQSGVPSRFSGSGSGTDFTLTISSLQPEDFATYYCQQSDSIPWTFGQGTKVEIK

SEQ ID NO: 74 - protein, 118 aa, Artificial Sequence
  VH of 5c8
QVQLVQSGAEVVKPGASVKLSCKASGYIFTSYYMYWVKQAPGQGLEWIGEINPSNGDTNFNEKFKSKATLTVDKSASTAYMELSSLRSEDTAVYYCTRSDGRNDMDSWGQGTLVTVSS

SEQ ID NO: 75 - protein, 111 aa, Artificial Sequence
  VL of 5c8
DIVLTQSPATLSVSPGERATISCRASQRVSSSTYSYMHWYQQKPGQPPKLLIKYASNLESGVPARFSGSGSGTDFTLTISSVEPEDFATYYCQHSWEIPPTFGGGTKLEIK

SEQ ID NO: 76 - DNA, 321 bp, Artificial Sequence
  cDNA of VH of C4LB231
gacatccagatgacccagagccccagcagcctgagcgccagcgtgggcgacagagtgaccatcacctgtcgggccagccagagcatcagcagctacctgaactggtatcagcagaagcccggcaaggcccccaagctgctgatctactacgccaacagcctgcagagcggcgtgcccagcagattcagcggcagcggctccggcaccgacttcaccctgaccatcagcagcctgcagcccgaggacttcgccacctactactgccagcagagcgacagcatcccctggaccttcggccagggcaccaaggtggaaatcaag

SEQ ID NO: 77 - DNA, 354 bp, Artificial Sequence
  cDNA of VL of C4LB231
caggtccagctggtgcagtctggcgccgaagtgaagaaacccggcagcagcgtgaaggtgtcctgcaaggccagcggcggcaccttcagcagctacggcatcagctgggtccgacaggccccaggacagggcctggaatggatgggctggatcagccccatcttcggcaacaccaactacgcccagaaattccagggcagagtgaccatcaccgccgacgagagcaccagcaccgcctacatggaactgagcagcctgcggagcgaggacaccgccgtgtactactgcgccagaagccggtactacggcgacctggactactggggccagggcaccctggtcaccgtgtcctct

SEQ ID NO: 78 - DNA, 387 bp, Artificial Sequence
  cDNA of VH of C4LB191
caggtgcagctggtgcagagcggcgctcaggtgcagctggtgcagtctggcgccgaagtgaagaaacctggcgccagcatgaaggtgtcctgcaaggccagcggctacaccttcaccgactactacatccactgggtgcgccaggccccaggccagggactggaatgggtgggacggttcaaccccaacagcggcgacaccaacggcgcccagaaattccagggcagagtgaccatgacccgggacaccagcatcagcaccgcctacatggaactgacccggctgcggagcgacgacaccgccgtgtaccactgtgccagagagggcgagctggccggcatcttcttcgactactggggccagggcaccctggtgacagtgtccagc

SEQ ID NO: 79 - DNA, 318 bp, Artificial Sequence
  cDNA of VL of C4LB191
agctacgagctgacccagccccccagcgtgtccgtgtctcctggccagaccgccagcatcacctgtagcggcgacaagctgggcgacaaatacgtgtcctggaaccaccagaagcccggccagagccccgtgctggtgatctaccaggaccggaagaggcccagcggcatccccgagagattcagcggcagcaacagcggcaacaccgccaccctgaccatcagcggcacccaggccatggacgaggccgactactactgccaggcctgggacagcagcaccgtggtgttcggcggaggcaccaagctgaccgtgctg

SEQ ID NO: 80 - protein, 448 aa, Artificial Sequence
  FL mAb C4LB89 VH on IgG1sigma
QVQLVQSGAEVKKPGSSVKVSCKASGGTFSSYGISWVRQAPGQGLEWMGWISPIFGNTNYAQKFQGRVTITADESTSTAYMELSSLRSEDTAVYYCARSRYYGDLDYWGQGTLVTVSSASTKGPSVFPLAPSSKSTSGGTAALGCLVKDYFPEPVTVSWNSGALTSGVHTFPAVLQSSGLYSLSSVVTVPSSSLGTQTYICNVNHKPSNTKVDKKVEPKSCDKTHTCPPCPAPEAAGASSVFLFPPKPKDTLMISRTPEVTCVVVDVSAEDPEVKFNWYVDGVEVHNAKTKPREEQYNSTYRVVSVLTVLHQDWLNGKEYKCKVSNKALPSSIEKTISKAKGQPREPQVYTLPPSREEMTKNQVSLTCLVKGFYPSDIAVEWESNGQPENNYKTTPPVLDSDGSFFLYSKLTVDKSRWQQGNVFSCSVMHEALHNHYTQKSLSLSPGK

SEQ ID NO: 81 - protein, 214 aa, Artificial Sequence
  Light chain of C4LB89
DIQMTQSPSSLSASVGDRVTITCRASQSISSYLNWYQQKPGKAPKLLIYYANSLQSGVPSRFSGSGSGTDFTLTISSLQPEDFATYYCQQSDSIPWTFGQGTKVEIKRTVAAPSVFIFPPSDEQLKSGTASVVCLLNNFYPREAKVQWKVDNALQSGNSQESVTEQDSKDSTYSLSSTLTLSKADYEKHKVYACEVTHQGLSSPVTKSFNRGEC

SEQ ID NO: 82 - protein, 448 aa, Artificial Sequence
  FL mAb C4LB89 VH on IgG1sigmaYTE
QVQLVQSGAEVKKPGSSVKVSCKASGGTFSSYGISWVRQAPGQGLEWMGWISPIFGNTNYAQKFQGRVTITADESTSTAYMELSSLRSEDTAVYYCARSRYYGDLDYWGQGTLVTVSSASTKGPSVFPLAPSSKSTSGGTAALGCLVKDYFPEPVTVSWNSGALTSGVHTFPAVLQSSGLYSLSSVVTVPSSSLGTQTYICNVNHKPSNTKVDKKVEPKSCDKTHTCPPCPAPEAAGASSVFLFPPKPKDTLYITREPEVTCVVVDVSAEDPEVKFNWYVDGVEVHNAKTKPREEQYNSTYRVVSVLTVLHQDWLNGKEYKCKVSNKALPSSIEKTISKAKGQPREPQVYTLPPSREEMTKNQVSLTCLVKGFYPSDIAVEWESNGQPENNYKTTPPVLDSDGSFFLYSKLTVDKSRWQQGNVFSCSVMHEALHNHYTQKSLSLSPGK

SEQ ID NO: 83 - protein, 444 aa, Artificial Sequence
  FL mAb C4LB89 VH on IgG2sigma
QVQLVQSGAEVKKPGSSVKVSCKASGGTFSSYGISWVRQAPGQGLEWMGWISPIFGNTNYAQKFQGRVTITADESTSTAYMELSSLRSEDTAVYYCARSRYYGDLDYWGQGTLVTVSSASTKGPSVFPLAPCSRSTSESTAALGCLVKDYFPEPVTVSWNSGALTSGVHTFPAVLQSSGLYSLSSVVTVPSSNFGTQTYTCNVDHKPSNTKVDKTVERKCCVECPPCPAPPAAASSVFLFPPKPKDTLMISRTPEVTCVVVDVSAEDPEVQFNWYVDGVEVHNAKTKPREEQFNSTFRVVSVLTVLHQDWLNGKEYKCKVSNKGLPSSIEKTISKTKGQPREPQVYTLPPSREEMTKNQVSLTCLVKGFYPSDIAVEWESNGQPENNYKTTPPMLDSDGSFFLYSKLTVDKSRWQQGNVFSCSVMHEALHNHYTQKSLSLSPGK

SEQ ID NO: 84 - protein, 119 aa, Artificial Sequence
  VH of C4LB119
QVQLVQSGAEVKKPGSSVKVSCKASGGTFSSYYISWVRQAPGQGLEWMGAIDPYFGYANYAQKFQGRVTITADESTSTAYMELSSLRSEDTAVYYCARTGLNYGGFDYWGQGTLVTVSS

SEQ ID NO: 85 - protein, 107 aa, Artificial Sequence
  VL of C4LB119
EIVLTQSPATLSLSPGERATLSCRASQSVSSYLAWYQQKPGQAPRLLIYDASNRATGIPARFSGSGSGTDFTLTISSLEPEDFAVYYCQQRSNWPLTFGQGTKVEIK

SEQ ID NO: 86 - protein, 121 aa, Artificial Sequence
  VH of C4LB83
QVQLVQSGAEVKKPGSSVKVSCKASGGTFSSYAISWVRQAPGQGLEWMGWIIPIFGNTNYAQKFQGRVTITADESTSTAYMELSSLRSEDTAVYYCAREKDFRGYTKLDYWGQGTLVTVSS

SEQ ID NO: 87 - protein, 107 aa, Artificial Sequence
  VL of C4LB83
DIQMTQSPSSLSASVGDRVTITCRASQSINNWLNWYQQKPGKAPKLLIYAASSLQSGVPSRFSGSGSGTDFTLTISSLQPEDFATYYCQQSFSFPYTFGQGTKVEIK